European Patent Application EP 4 600 266 A1, published August 13, 2025. Title: CHIMERIC ANTIGEN RECEPTOR TARGETING CD5 AND IMMUNE CELLS EXPRESSING SAME. Applicant: GC CELL CORPORATION. Application EP 23875185.3, filed October 4, 2023. The sequence listing filed with the application follows.

SEQUENCE LISTING (40 sequences)

SEQ ID NO: 1 - DNA, 63 bp, synthetic construct
  source 1..63: mol_type = other DNA
atggccttaccagtgaccgccttgctcctgccgctggccttgctgctccacgccgccaggccg

SEQ ID NO: 2 - DNA, 63 bp, synthetic construct
  source 1..63: mol_type = other DNA
atggctctgccagtgactgcactgctgctgccactggccctgctgctgcacgcagctcgacct

SEQ ID NO: 3 - protein, 21 aa, synthetic construct
MALPVTALLLPLALLLHAARP

SEQ ID NO: 4 - DNA, 720 bp, synthetic construct
  source 1..720: mol_type = other DNA
gacatccagatgacccagagccccagcagcctgagcgccagcgtgggcgacagagtgaccatcacctgcaaggccagccaggacatcaacagctacctgagctggttccagcagaagcccggcaaggcccccaagaccctgatctacagagccaacagactggtggacggcgtgcccagcagattcagcggcagcggcagcggccaggactacaccctgaccatcagcagcctgcagcccgaggacttcgccacctactactgcctgcagtacgacgagttcccctggaccttcggccagggcaccaaggtggagatcaagggtggcggtggatcgggcggtggtggatctggaggaggtggctcccaggtgcagctggtgcagagcggcagcgagctgaagaagcccggcgccagcgtgaaggtgagctgcaaggccagcggctacaccttcaccaactacggcgtgaactgggtgagacaggcccccggccagggcctggagtggatgggctggatcaacacccacaccggcgagcccacctacgccgaggagttcaagggcagattcgtgttcagcctggacaccagcgtgagcaccgcctacctgcagatcagcagcctgaaggccgaggacaccgccgtgtactactgcgccagagacgactactacgtgagagtggactactggggccagggcaccaccgtgaccgtgagcagc

SEQ ID NO: 5 - protein, 240 aa, synthetic construct
DIQMTQSPSSLSASVGDRVTITCKASQDINSYLSWFQQKPGKAPKTLIYRANRLVDGVPSRFSGSGSGQDYTLTISSLQPEDFATYYCLQYDEFPWTFGQGTKVEIKGGGGSGGGGSGGGGSQVQLVQSGSELKKPGASVKVSCKASGYTFTNYGVNWVRQAPGQGLEWMGWINTHTGEPTYAEEFKGRFVFSLDTSVSTAYLQISSLKAEDTAVYYCARDDYYVRVDYWGQGTTVTVSS

SEQ ID NO: 6 - DNA, 720 bp, synthetic construct
  source 1..720: mol_type = other DNA
gaaattcagctggtgcagagcggcggcggcctggtgaaaccgggcggcagcgtgcgcattagctgcgcggcgagcggctatacctttaccaactatggcatgaactgggtgcgccaggcgccgggcaaaggcctggaatggatgggctggattaacacccataccggcgaaccgacctatgcggatagctttaaaggccgctttacctttagcctggatgatagcaaaaacaccgcgtatctgcagattaacagcctgcgcgcggaagataccgcggtgtatttttgcacccgccgcggctatgattggtattttgatgtgtggggccagggcaccaccgtgaccgtgagcagcggtggcggtggctcgggcggtggtgggtcgggtggcggcggatctgatattcagatgacccagagcccgagcagcctgagcgcgagcgtgggcgatcgcgtgaccattacctgccgcgcgagccaggatattaacagctatctgagctggtttcagcagaaaccgggcaaagcgccgaaaaccctgatttatcgcgcgaaccgcctggaaagcggcgtgccgagccgctttagcggcagcggcagcggcaccgattataccctgaccattagcagcctgcagtatgaagattttggcatttattattgccagcagtatgatgaaagcccgtggacctttggcggcggcaccaaactggaaattaaa

SEQ ID NO: 7 - protein, 240 aa, synthetic construct
EIQLVQSGGGLVKPGGSVRISCAASGYTFTNYGMNWVRQAPGKGLEWMGWINTHTGEPTYADSFKGRFTFSLDDSKNTAYLQINSLRAEDTAVYFCTRRGYDWYFDVWGQGTTVTVSSGGGGSGGGGSGGGGSDIQMTQSPSSLSASVGDRVTITCRASQDINSYLSWFQQKPGKAPKTLIYRANRLESGVPSRFSGSGSGTDYTLTISSLQYEDFGIYYCQQYDESPWTFGGGTKLEIK

SEQ ID NO: 8 - DNA, 144 bp, synthetic construct
  source 1..144: mol_type = other DNA
gcgaagcccaccacgacgccagcgccgcgaccaccaacaccggcgcccaccatcgcgtcgcagcccctgtccctgcgcccagaggcgtgccggccagcggcggggggcgcagtgcacacgagggggctggacttcgcctgtgat

SEQ ID NO: 9 - DNA, 144 bp, synthetic construct
  source 1..144: mol_type = other DNA
gcaaaacctaccacaactcctgcaccacgcccccctactccagcacctaccatcgcatctcagccactgagtctgcgaccagaggcctgccggcccgccgccggcggggccgtccataccagagggctggactttgcctgcgat

SEQ ID NO: 10 - protein, 48 aa, synthetic construct
AKPTTTPAPRPPTPAPTIASQPLSLRPEACRPAAGGAVHTRGLDFACD

SEQ ID NO: 11 - DNA, 204 bp, synthetic construct
  source 1..204: mol_type = other DNA
ttttgggtgctggtggtggttggtggagtcctggcttgctatagcttgctagtaacagtggcctttattattttctgggtgaggagtaagaggagcaggctcctgcacagtgactacatgaacatgactccccgccgccccgggcccacccgcaagcattaccagccctatgccccaccacgcgacttcgcagcctatcgctcc

SEQ ID NO: 12 - DNA, 204 bp, synthetic construct
  source 1..204: mol_type = other DNA
ttctgggtactggtggttgtgggcggcgttctggcttgctattcactcctcgttacggttgcatttataatattttgggtacgctcaaagcgctcaagattgctccattctgattacatgaacatgacccctcgccggccgggtcccactcgcaaacactaccaaccttatgcccctccgcgggatttcgcggcctacaggtca

SEQ ID NO: 13 - protein, 68 aa, synthetic construct
FWVLVVVGGVLACYSLLVTVAFIIFWVRSKRSRLLHSDYMNMTPRRPGPTRKHYQPYAPPRDFAAYRS

SEQ ID NO: 14 - DNA, 66 bp, synthetic construct
  source 1..66: mol_type = other DNA
gaaagggtccaacccctggaagagaatgtgggaaatgcagccaggccaagattcgagaggaacaag

SEQ ID NO: 15 - DNA, 66 bp, synthetic construct
  source 1..66: mol_type = other DNA
gagagagtacaacctcttgaggagaatgtcggcaacgctgccaggccgcggtttgagcgaaataag

SEQ ID NO: 16 - protein, 22 aa, synthetic construct
ERVQPLEENVGNAARPRFERNK

SEQ ID NO: 17 - DNA, 336 bp, synthetic construct
  source 1..336: mol_type = other DNA
agagtgaagttcagcaggagcgcagacgcccccgcgtaccagcagggccagaaccagctctataacgagctcaatctaggacgaagagaggagtacgatgttttggacaagagacgtggccgggaccctgagatggggggaaagccgagaaggaagaaccctcaggaaggcctgtacaatgaactgcagaaagataagatggcggaggcctacagtgagattgggatgaaaggcgagcgccggaggggcaaggggcacgatggcctttaccagggtctcagtacagccaccaaggacacctacgacgcccttcacatgcaggccctgccccctcgc

SEQ ID NO: 18 - DNA, 336 bp, synthetic construct
  source 1..336: mol_type = other DNA
cgagtcaagttttctcgaagtgccgacgctcctgcctatcagcaaggccagaatcaactgtataacgagcttaacttgggccggagggaggagtacgatgtgctggataagcgcaggggacgggacccggaaatgggcggaaagcccaggcggaaaaacccacaggaaggactctacaatgaactccaaaaggacaaaatggcagaggcctattcagagattgggatgaagggagaaaggaggcgaggaaaagggcacgacggcttgtatcagggcttgtctacggccactaaagacacctatgatgccctgcatatgcaggcacttccccccaga

SEQ ID NO: 19 - protein, 112 aa, synthetic construct
RVKFSRSADAPAYQQGQNQLYNELNLGRREEYDVLDKRRGRDPEMGGKPRRKNPQEGLYNELQKDKMAEAYSEIGMKGERRRGKGHDGLYQGLSTATKDTYDALHMQALPPR

SEQ ID NO: 20 - DNA, 54 bp, synthetic construct
  source 1..54: mol_type = other DNA
gaaggccgaggttcattgctcacctgtggcgatgtggaagaaaatccaggtccg

SEQ ID NO: 21 - protein, 18 aa, synthetic construct
EGRGSLLTCGDVEENPGP

SEQ ID NO: 22 - DNA, 486 bp, Homo sapiens
  source 1..486: mol_type = genomic DNA
atgagaatttcgaaaccacatttgagaagtatttccatccagtgctacttgtgtttacttctaaacagtcattttctaactgaagctggcattcatgtcttcattttgggctgtttcagtgcagggcttcctaaaacagaagccaactgggtgaatgtaataagtgatttgaaaaaaattgaagatcttattcaatctatgcatattgatgctactttatatacggaaagtgatgttcaccccagttgcaaagtaacagcaatgaagtgctttctcttggagttacaagttatttcacttgagtccggagatgcaagtattcatgatacagtagaaaatctgatcatcctagcaaacaacagtttgtcttctaatgggaatgtaacagaatctggatgcaaagaatgtgaggaactggaggaaaaaaatattaaagaatttttgcagagttttgtacatattgtccaaatgttcatcaacacttct

SEQ ID NO: 23 - DNA, 486 bp, synthetic construct
  source 1..486: mol_type = other DNA
atgcgcataagtaagcctcatctgcggtccatttctatacaatgttatctgtgcttgcttttgaactcccactttcttacggaagcaggcattcatgtgttcattctgggttgtttttctgccgggctgcccaaaaccgaggccaactgggtcaacgtgatcagcgacctcaagaagatcgaggatttgattcaaagtatgcatatagacgccacactctatactgagtccgacgttcacccgagttgtaaagttacggctatgaagtgctttttgttggaactccaggtgatttcccttgaatccggcgatgcgagcatccacgatacggtagagaatcttattattctggcgaataattctctgtcttcaaatgggaatgtaactgagagcggttgtaaagaatgcgaagaacttgaagaaaagaatatcaaggaatttcttcagagtttcgtgcatattgttcaaatgttcatcaacacatcc

SEQ ID NO: 24 - protein, 162 aa, Homo sapiens
MRISKPHLRSISIQCYLCLLLNSHFLTEAGIHVFILGCFSAGLPKTEANWVNVISDLKKIEDLIQSMHIDATLYTESDVHPSCKVTAMKCFLLELQVISLESGDASIHDTVENLIILANNSLSSNGNVTESGCKECEELEEKNIKEFLQSFVHIVQMFINTS

SEQ ID NO: 25 - DNA, 15 bp, synthetic construct
  source 1..15: mol_type = other DNA
aactatggcatgaac

SEQ ID NO: 26 - protein, 5 aa, synthetic construct
NYGMN

SEQ ID NO: 27 - DNA, 51 bp, synthetic construct
  source 1..51: mol_type = other DNA
tggattaacacccataccggcgaaccgacctatgcggatagctttaaaggc

SEQ ID NO: 28 - protein, 17 aa, synthetic construct
WINTHTGEPTYADSFKG

SEQ ID NO: 29 - DNA, 27 bp, synthetic construct
  source 1..27: mol_type = other DNA
cgcggctatgattggtattttgatgtg

SEQ ID NO: 30 - protein, 9 aa, synthetic construct
RGYDWYFDV

SEQ ID NO: 31 - DNA, 354 bp, synthetic construct
  source 1..354: mol_type = other DNA
gaaattcagctggtgcagagcggcggcggcctggtgaaaccgggcggcagcgtgcgcattagctgcgcggcgagcggctatacctttaccaactatggcatgaactgggtgcgccaggcgccgggcaaaggcctggaatggatgggctggattaacacccataccggcgaaccgacctatgcggatagctttaaaggccgctttacctttagcctggatgatagcaaaaacaccgcgtatctgcagattaacagcctgcgcgcggaagataccgcggtgtatttttgcacccgccgcggctatgattggtattttgatgtgtggggccagggcaccaccgtgaccgtgagcagc

SEQ ID NO: 32 - protein, 118 aa, synthetic construct
EIQLVQSGGGLVKPGGSVRISCAASGYTFTNYGMNWVRQAPGKGLEWMGWINTHTGEPTYADSFKGRFTFSLDDSKNTAYLQINSLRAEDTAVYFCTRRGYDWYFDVWGQGTTVTVSS

SEQ ID NO: 33 - DNA, 33 bp, synthetic construct
  source 1..33: mol_type = other DNA
cgcgcgagccaggatattaacagctatctgagc

SEQ ID NO: 34 - protein, 11 aa, synthetic construct
RASQDINSYLS

SEQ ID NO: 35 - DNA, 21 bp, synthetic construct
  source 1..21: mol_type = other DNA
cgcgcgaaccgcctggaaagc

SEQ ID NO: 36 - protein, 7 aa, synthetic construct
RANRLES

SEQ ID NO: 37 - DNA, 27 bp, synthetic construct
  source 1..27: mol_type = other DNA
cagcagtatgatgaaagcccgtggacc

SEQ ID NO: 38 - protein, 9 aa, synthetic construct
QQYDESPWT

SEQ ID NO: 39 - DNA, 321 bp, synthetic construct
  source 1..321: mol_type = other DNA
gatattcagatgacccagagcccgagcagcctgagcgcgagcgtgggcgatcgcgtgaccattacctgccgcgcgagccaggatattaacagctatctgagctggtttcagcagaaaccgggcaaagcgccgaaaaccctgatttatcgcgcgaaccgcctggaaagcggcgtgccgagccgctttagcggcagcggcagcggcaccgattataccctgaccattagcagcctgcagtatgaagattttggcatttattattgccagcagtatgatgaaagcccgtggacctttggcggcggcaccaaactggaaattaaa

SEQ ID NO: 40 - protein, 107 aa, synthetic construct
DIQMTQSPSSLSASVGDRVTITCRASQDINSYLSWFQQKPGKAPKTLIYRANRLESGVPSRFSGSGSGTDYTLTISSLQYEDFGIYYCQQYDESPWTFGGGTKLEIK